European Patent Application EP 4 621 066 A1, published September 24, 2025. Title: MULTI-TEMPLATE NUCLEIC ACID SYNCHRONOUS SEQUENCING METHOD AND USE THEREOF. Applicant: MGI TECH CO., LTD. The sequence listing filed with the application follows.

SEQUENCE LISTING (2 sequences)

SEQ ID NO: 1 - DNA, 94 bp, synthetic construct
  source 1..94: mol_type = other DNA
cgccgacgcacagggtgcctcgaccgcatggcgcggaaccatggttccgcgccaactccttggctcacagaacgacatggctacgatccgactt

SEQ ID NO: 2 - DNA, 94 bp, synthetic construct
  source 1..94: mol_type = other DNA
catgcggtcgaggcaccctgtgcgtcggcgggctgcatgccggcatgcagcccaactccttggctcacagaacgacatggctacgatccgactt